European Patent Application EP 4 394 035 A1, published July 3, 2024. Title: LIPASE MUTANT AND APPLICATION THEREOF. Applicant: ASYMCHEM LIFE SCIENCE (TIANJIN) CO., LTD. The sequence listing filed with the application follows.

SEQUENCE LISTING (2 sequences)

SEQ ID NO: 1 - protein, 381 aa, Pseudomonas putida
MQIQGHYELKFEAVRETFAALFDDPQERGAALCIQVGGETVVDLWAGSADKDGQQAWHSDTIANLFSCTKTFTAVTALQLVGEGKLTLDAPVANYWPEFAQAGKQAITLRQLLSHRAGLPAIRELLPAEALYDWQAMVDALAAETPWWTPGTEHGYAAITYGWLIGELIRRADGRGPGDSIVARTARPLGLDFHVGLADDEFYRVAHIARGKGNAGDAAAQRLLQVTMREPEALSTRAFTNPPAILTSTNKPEWRRMQQPAANGHGNARSLAGFYAGLLDGSLLESELLDELTREHSLGQDRTLLTQTRFGLGCMLDQPDVANATFGLGARAFGHPGAGGSVGFADPEHDVAFGFVVNTLGPYVLMDPRAQKLVRVLASCL

SEQ ID NO: 2 - DNA, 1143 bp, Pseudomonas putida
atgcagatccaaggccactatgagctgaagttcgaggcagtgcgcgagacgttcgcagcgctgttcgacgacccgcaagagcgtggtgctgcactgtgtatccaggtcggtggcgaaaccgtagtcgacctgtgggcaggtagcgcagataaggacggtcagcaagcgtggcatagcgacaccatcgcaaacctgttctcctgcaccaaaaccttcaccgcggttaccgctctgcagctggtgggcgaaggcaaactgaccctggacgcgcctgtggcaaactactggccagaattcgcgcaggcaggtaaacaggctatcactctgcgccagctgctgagccaccgtgccggtctgccagcaatccgtgaactgctgccggctgaagcactgtacgactggcaagcaatggtggatgccctggcagcagaaaccccgtggtggactccgggtactgaacatggttacgccgctattacctacggctggctgatcggcgaactgatccgtcgtgcggacggtcgtggtcctggtgactctattgtggcccgtactgctcgtccgctgggtctggatttccatgtcggtctggccgatgacgaattctatcgcgttgcgcacattgcgcgtggcaaaggcaacgcgggcgatgctgcggctcagcgtctgctgcaggttactatgcgtgaaccggaagctctgtctacccgtgctttcaccaacccgccggcgattctgacttccacgaacaaaccggaatggcgccgtatgcagcagccggcggctaacggtcacggtaatgctcgctctctggctggtttttacgcgggtctgctggacggtagcctgctggaatctgagctgctggatgaactgacgcgcgaacactccctgggccaggatcgcaccctgctgacccagactcgctttggtctgggttgtatgctggaccagccggatgttgctaatgccacgtttggcctgggcgcgcgtgcgttcggccacccaggcgcgggcggctctgttggcttcgctgatccggaacacgatgttgcgtttggctttgttgtaaacaccctgggtccgtatgttctgatggatccgcgtgcccagaaactggtacgtgtactggcctcctgcctg